European Patent Specification EP 3 786 291 B1, published October 18, 2023. Title: Amadoriase with improved dehydrogenase activity. Applicant: Kikkoman Corporation. Application PCT/JP2015/080014. The sequence listing filed with the application follows.

SEQUENCE LISTING (82 sequences)

SEQ ID NO: 1 - protein, 437 aa, Coniochaeta sp. [sequence omitted]

SEQ ID NO: 2 - DNA, 1314 bp, Coniochaeta sp.
atgacgtcgaatcgtgcagatacaagggtgattgtcgtcggtggcggaggaacgattggttcctcgacagcgctgcatcttgtgaggagtggttatgctcccgcaaatatcacggtcttggacacatttgagattccatcggctcaatcagccggccatgatctcaacaagatcatgggaatacgactgcgcaacaaggtggacctgcaaatgagtctagaggctagacagatgtggaaggaggatgagttattccagcccttctttcacaataccggcagaatggactgcgaacacacgcctgagggtatcgaggacctgaaaaagcagtaccaggcactgcacgatgccggtgcgggtctggagaagactcatgcctggttggacaacgaggatgagatcttatccaagatgccgttgcttcaacgtgaccaaatacaaggatggaaagcaatatggagtcaagatggcggctggttagctgcggcaaaggccatcaatgcgatcggacagttcttgaaagaacgtggtgtaaagttcggattcggcggcgctggatccttcaagcaaccccttttcgacgatgaaggcacaacttgcattggcgttgagacggcagatggtaccaaatattacgctgacaaggtggtcttagcagctggcgcatggagcccaaccctggtggacctggaagatcaatgttgctcgaaggcttgggtgtatgctcatattcagttgacgcctgaagaggccgctgagtataagggtgtcccagttgtgtataatggcgaatttggcttcttctttgagcctgatgagtttggtgtaataaaggtgtgcgacgagttcccaggattctcgcgcttcaaggaacatcaaccctatggcgccccatctccgaaacggatatcagtaccacgatcgcacgccaagcatcccacagacacttatccagacgcatccgaagtcagcatcaaaaaagcaatcgcgacgtttctccctcgatttcaggacaaggagctcttcaatcgcgccttgtgctggtgtacagacactgcggacgctgctctcttgatgtgtgaacaccccaaatggaagaatttcattctagcgaccggcgacagcggacactcattcaaaatcttgcctaacgtcggaaaatacgtagtcgagttgatagagggccgcctgccggaggaaatggcttatcaatggaggtggcggccaggaggcgatgcactcaagtctagacgtgcggcaccgccaaaagatcttgcagacatgccaggatggaaacatgatccgaaattgtaa

SEQ ID NO: 3 - protein, 437 aa, Eupenicillium terrenum
MAHSRASTKVVVVGGGGTIGSSTALHLIRSGYTPSNITVLDVYKTPSLQSAGHDLNKIMGIRLRNGPDLQLSLESLDMWQNDELFKPFFHQVGMIDCSSSKEGIENLRRKYQTLLDAGIGLEKTNVWLESEDEILAKAPNFTREQVKGWKGLFCTDGGWLAAAKAINAIGIFLQDKGVKFGFGGAGTFQQPLFAADGKTCIGLETTDGTKYFADKVVLAAGAWSPTLVDLEDQCVSKAWVFAHIQLTPKEADAYKNVPVVYDGEYGFFFEPNEYGVIKVCDEFPGFSRFKLHQPYGAASPKMISVPRSHAKHPTDTYPDASEVTIRKAIARFLPEFKDKELFNRTMCWCTDTADANLLICEHPKWKNFILATGDSGHSFKLLPNIGKHVVELLEGSLSQEMAGAWRWRPGGDALRSRRGAPAKDLAEMPGWKHDAHL

SEQ ID NO: 4 - protein, 440 aa, Pyrenochaeta sp.
MAASRAKTTVIVVGGGGTIGSSTALHLLRSGYTPSNITVLDTYPIPSLQSAGNDLNKIMGIRLRNKVDLQLSLEAREMWREDELFRDFFHNTGRLDCAHGEKGINDLRQAYQTLLDANAGLEETNEWLDSEDEILARMPLLSREQIKGWKAVFSRDGGWLAAGKAINAIGEYLRKEGVKFGFGGAGSFQQPLLAEGICIGVETTDGTRYYADKVVLAAGAWSPALVDLEDQCVSKAWVYAHMQLTPKEAAAYKDTPVVYNGDLGFFFEPNEHGVIKVCDEFPGFTRFKKHQPFGARAPKRISVPRSHAKHPTDTYPHASEASIKKAIAAFLPQFKDKELFNRAMCWCTDTADAALLICEHPQWKNFMLATGDSGHSFKLLPNIGKHVVELIEGTLAADLAHAWRWRPGIGDALQSRRAAPAKDLADMPGWNHDESPRAKL

SEQ ID NO: 5 - protein, 452 aa, Arthrinium sp.
MAASRKTTKVIVVGGGGTIGSSTALHLLRSGYTATNITVLDTYPIPSAQSAGNDLNKIMGIRLRNPVDKQLSLEAQDMWCHDELFKPYFHNTGRMDCEGTEKGIAALKQQYQTLLDADVGLEKTTEWLDSEDAILAKMPLLERDQIKGWKAIFSQDGGWLAAAKAINAIGEELKRQGVNFGFGGAGAFKKPLFAPDGSTCIGVETVDGTKYYGDKVVLAAGAWSPALVDLEEQCCSKAWVYAHMQLTPHEAAEYQGCPVVYHGDLGFFFEPNEHGVIKVCDEFPGFTRFLEQHQSYGAPAPTRVSVPRSHAKHPTDTYPDASEQSIRRAVAAFLPRFQSKELFNRAMCWCTDTADAALLICEHPRWRNFILATGDSGHSFKLLPNIGKHVVELLEGRLADDLAQAWRWRPGQGDALKSRRAAPAKDLADMPGWNHDGDSGNATSGTSSEHKL

SEQ ID NO: 6 - protein, 440 aa, Curvularia clavata
MAPSRANTSVIVVGGGGTIGSSTALHLVRSGYTPSNITVLDTYPIPSAQSAGNDLNKIMGIRLRNKVDLQLSLEARQMWREDDLFKEYFHNTGRLDCAHGEEGLADLRQAYQALLDANAGLEETTEWLDSEDEILKKMPLLDREQIKGWKAVYSQDGGWLAAAKAINAIGEYLRAQGVKFGFGGAGSFKQPLLAEGVCIGVETVDGTRYYADKVVLAAGAWSPVLVDLEDQCVSKAWVYAHIQLTPEEAAEYKNVPVVYNGDVGFFFEPDEHGVIKVCDEFPGFTRFKQHQPYGAKAPKRISVPRSAAKHPTDTYPDASEKSIRKAIATFLPKFTEKELFNRHLCWCTDTADAALLMCEHPEWKNFVLATGDSGHTFKLLPNIGKHVVELLEGTLAEDLAHAWRWRPGTGDALKSRRAAPAKDLADMPGWKHDDVVKSKL

SEQ ID NO: 7 - protein, 441 aa, Neocosmospora vasinfecta
MTTPRKETTVLIIGGGGTIGSSTALHLLRAGYTPSNITVLDTYPIPSAQSAGNDLNKIMGIRLRNKVDLQLSLEARDMWRNDALFRPFFHNTGRLDCESSAEGVEGLRREYQKLVEAGVGLEETHEWLDSEEAILEKAPLLQREEIEGWKAIWSEEGGWLAAAKAINAIGEELQRQGVRFGFGGAGSFKRPLFADDGTTCIGVETVDGTQYHADKVVLAAGAWSPALVDLEEQCCSKAWVYAHMQLTPEEAAVYKGCPVVYHGDVGFFFEPNENGVIKVCDEFPGFTRFKQHQPYGAPAPKPVSVPRSHAKHPTDTYPDASEESIKRAVSTFLPRFKDKPLFNRALCWCTDTADSALLICEHPRWKNFILATGDSGHSFKLLPIIGKHVVELVEGRLADDLAEAWRWRPGQGDARKSIRAAPAKDLADMPGWKHDQDSESR

SEQ ID NO: 8 - protein, 477 aa, Cryptococcus neoformans
MPPSRASTKVIVIGGGGTLGSSTALHLLRAGYTPSNITVLDTYLIPSAQSAGNDLNKIMGIRIRNPVDKQLSLEARDMWRNDEVFKPYFHNTGRLDCAHTPESIASLRKSYEAILKAGSGLEKTHHWLSTEDEILARAPLLDRKQIKGWKAIYSEDGGWLAAAKAINSIGQVLKEKGVTFGFGSAGSFKKPLFDEDGTKAIGIETVDGTQYFADKVVLAAGAWSPTLVDLEGQCCSKAWVYAHMQLTPEEAAEYKECPVVYNSELGFFFEPNEKGVIKVCDEFPGFTRFKQHQPYGASSTKHISFPRSHAKHPTDTIPDESDASIRRAISAFLPRFKEKELFNRALCWCTDTADANLLICEHPKWKNFILATGDSGHSFKILPNIGKHVVELIEGTLAEDLAESWRWRPGSGDPLISRRAAPARDLADLPGWNHDEPSDDDMDVKDVAVSLASVKIGENIGEKVVEDGARVGVKVLA

SEQ ID NO: 9 - protein, 437 aa, Phaeosphaeria nodorum
MAPSRANTSVIVVGGGGTIGSSTALHLVRSGYTPSNVTVLDAYPIPSSQSAGNDLNKIMGVSLRNPVDLQLALEARQMWNEDELFKKFFHNTGRLDCAHGEKDIADLKSGYQALVDAGLDATNEWLDSEDEILKRMPLLSRDQIKGWKAIFSKDGGWLAAAKAINAVGEYLRDQGVRFGFYGAGSFKAPLLAEGVCIGVETVDGTRYYADKVVLAAGAWSPTLVELHEQCVSKAWVYGHIQLTPEEAARYKNSPVVYNGDVGFFFEPNEHGVIKVCDEFPGFTRFKMHQPFGAKAPKRISVPRSHAKHPTDTIPDASDVSIRRAIATFMPQFKNKKMFNQAMCWCTDTADAALLICEHPEWKNFVLATGDSGHSFKLLPNIGKHVVELLEGTLADDLAHAWRWRPGSGDALKSRRSAPAKDLADMPGWNHDKPRANL

SEQ ID NO: 10 - protein, 438 aa, Aspergillus nidulans
MTPRANTKIIVVGGGGTMGSSTALHLLRAGYTPSNITVLDTCPIPSAQSAGYDLNKIMSIRLRNKPDLQLSLEALDMWKNDPLFKPFFHNVGMIDVSSTEEGIEGLRKKYQSLLDAGIGLEKTNFMLESEDEILAKAPHFTQEQIKGWKGLFCGDGGWLAAAKAINAIGQFLKEQGVKFGFGGAGTFKKPLFADAHEKTCIGVETVDGTKYYADKVVLAAGAWSSTLVDLEEQCVSKAWVFAHIQLTPAEAAAYKNTPVIYDGDYGFFFEPNENGIIKVCDEFPGFTHFKMHQPYGSPAPKPISVPRSHAKHPTDTYPHASEVTIKKAINRFLPRFNDKELFNRAMCWCTDTADANLLVCEHPRWKGFYLATGDSGHSFKLLPNIGKHVVELLEERLESVFKDAWRWRPGSGDALKSRRAAPAKDLADMPGWRNEAKM

SEQ ID NO: 11 - protein, 438 aa, Emericella nidulans
MAPRANTKIIVVGGGGTMGSSTALHLLRAGYTPSNITVLDTYPIPSAQSAGYDLNKIFGIRLRNKPDLQLYLEALDMWKNDPLFKPFFHNVGQMDVSSTEEGIKKLRMRYQSLLDAGIGLEKTNFLLESEDEILAKAPHFTREQIKGWKGLFCGDGGWLAAAKAINAIGQFLKEQGVKFGFGEAGTFKKPLFADADEKTCIGVETVDGTKYYADKVVLAAGAWSSTLVDLEEQCVSKAWVFAHIQLTPAEAAAYKNTPVIYDGDYGFFIEPDENGIIKVCDEFPGFTHFKMHQPYGSPVPKLISVPRSHAKHPTDTYPHASEVTIKKAINRFLPRFNDKELFNRAMCWCTDTADANLLVCEHPRWKGFYLATGDSGHSFKLLPNIGKHVVELLEGRLESVFKDAWRWRPGSGDALKSRRAAPAKDLADMPGWRNEAKM

SEQ ID NO: 12 - protein, 441 aa, Ulocladium sp.
MAPNRANISVIVVGGGGTIGSSTALHLVRSGYTPSNITVLDTYPIPSAQSAGNDLNKIMGIRLRNKVDLQLSLEARQMWTEDDLFKEYFHKTGRLDCAHGEKGLADLKQAYQALLDANAGLEATTEWLDSEDKILEKMPLLNRDQIKGWKAVFSEDGGWLAAAKAINAIGRFLRDQGVKFGFGGAGSFKQPLLAEGVCVGVETVDGTRYYADKVVLAAGAWSPALVDLQDQCVSKAWVYAHIQLSPSEAAEYKNVPVVYNGDVGFFFEPDEYGVIKVCDEFPGFTRFKQHQPFGASAPKRISVPRSAAKHPTDTYPDASEVSIRKAIATFLPKFTEKEVFNRHLCWCTDTADAALLMCEHPEWKNFVLATGDSGHTFKLLPNIGKHVVELLEGTLADDLAHAWRWRPGTGDALKSRRAARAKDLADMPGWNHDGEAPRAKL

SEQ ID NO: 13 - protein, 437 aa, Penicillium janthinellum
MAHSRESTKIVIVGGGGTMGSSTALHLIRSGYTPSNITVLDVYPIPSLQSAGYDLNKIMSIRLRNGPDLQLSLEALDMWKNDPLFKPFFHNVGMLDCSSSQEGIASLRRKHQDLIDANIGLEKTNIWLESEDDILAKAPHFTREQIKGWKGLFCGDGGWLAAAKAINAIGTFLKSQGVKFGFGSAGTFKRPLFAPDGATCSGVETVDGTKYFADKVVLAAGAWSSTLVDLEDQCVSKAWVFAHIQLTPQESAQYKDVPVVYDGDYGFFFEPNEHGVIKVCDEFPGFSRFKLHQPYGATSPKLISVPRSHAKHPTDTYPDSSEETIRKAIARFMPRFKDKELFNRSMCWCTDTADANLLICEHPKWKNFILATGDSGHSFKVLPNIGKHVVELIEGRLPQDLAGAWRWRPGGDALKSKRSAPAKDLAEMPGWKHDAKL

SEQ ID NO: 14 - DNA, 30 bp, Artificial
  primer
gtaataaaggtgcaggacgaattcccagga

SEQ ID NO: 15 - DNA, 27 bp, Artificial
  primer
gaagcgcgagaatcctgggaattcgtc

SEQ ID NO: 16 - DNA, 30 bp, Artificial
  primer
gtaataaaggtgagcgacgaattcccagga

SEQ ID NO: 17 - DNA, 30 bp, Artificial
  primer
gtaataaaggtggatgacgaattcccagga

SEQ ID NO: 18 - DNA, 30 bp, Artificial
  primer
gtaataaaggtggaagacgaattcccagga

SEQ ID NO: 19 - DNA, 30 bp, Artificial
  primer
gtaataaaggtgatggacgaattcccagga

SEQ ID NO: 20 - DNA, 30 bp, Artificial
  primer
gtaataaaggtgaaagacgaattcccagga

SEQ ID NO: 21 - DNA, 30 bp, Artificial
  primer
gtaataaaggtgcgtgacgaattcccagga

SEQ ID NO: 22 - DNA, 30 bp, Artificial
  primer
gtaataaaggtggtggacgaattcccagga

SEQ ID NO: 23 - DNA, 30 bp, Artificial
  primer
gtaataaaggtgaacgacgaattcccagga

SEQ ID NO: 24 - DNA, 30 bp, Artificial
  primer
ggcgaatttggctatttcttcgaacctgat

SEQ ID NO: 25 - DNA, 30 bp, Artificial
  primer
tattacaccaaactcatcaggttcgaagaa

SEQ ID NO: 26 - DNA, 27 bp, Artificial
  primer
ggcttcttctatgaacctgatgagttt

SEQ ID NO: 27 - DNA, 27 bp, Artificial
  primer
ctttattacaccaaactcatcaggttc

SEQ ID NO: 28 - DNA, 30 bp, Artificial
  primer
tcagccggccataacctcaacaagatcatg

SEQ ID NO: 29 - DNA, 30 bp, Artificial
  primer
gcgcagtcgtattcccatgatcttgttgag

SEQ ID NO: 30 - DNA, 30 bp, Artificial
  primer
tcagccggccatgcgctcaacaagatcatg

SEQ ID NO: 31 - DNA, 30 bp, Artificial
  primer
aaggcttgggtggaagctcatattcagttg

SEQ ID NO: 32 - DNA, 30 bp, Artificial
  primer
ggcctcttcaggcgtcaactgaatatgagc

SEQ ID NO: 33 - DNA, 30 bp, Artificial
  primer
aaggcttgggtgcaggctcatattcagttg

SEQ ID NO: 34 - DNA, 30 bp, Artificial
  primer
aaggcttgggtgaaagctcatattcagttg

SEQ ID NO: 35 - DNA, 30 bp, Artificial
  primer
cacctttattacaccaaactcatcaggctc

SEQ ID NO: 36 - DNA, 30 bp, Artificial
  primer
tgtaataaaggtgcacgacgagttcccagg

SEQ ID NO: 37 - DNA, 30 bp, Artificial
  primer
tgtaataaaggtgaccgacgagttcccagg

SEQ ID NO: 38 - DNA, 30 bp, Artificial
  primer
gccaaattcgccattatacacaactgggac

SEQ ID NO: 39 - DNA, 30 bp, Artificial
  primer
ttattctttgagcctgatgagtttggtgta

SEQ ID NO: 40 - DNA, 30 bp, Artificial
  primer
atgttctttgagcctgatgagtttggtgta

SEQ ID NO: 41 - DNA, 30 bp, Artificial
  primer
gaagaagccaaattcgccattatacacaac

SEQ ID NO: 42 - DNA, 30 bp, Artificial
  primer
ttagagcctgatgagtttggtgtaataaag

SEQ ID NO: 43 - DNA, 30 bp, Artificial
  primer
atggagcctgatgagtttggtgtaataaag

SEQ ID NO: 44 - protein, 437 aa, Eupenicillium terrenum
MAHSRASTKVVVVGGGGTIGSSTALHLIRSGYTPSNITVLDVYKTPSLQSAGHDLNKIMGIRLRNGPDLQLSLESLDMWQNDELFKPFFHQVGMIDCSSSKEGIENLRRKYQTLLDAGIGLEKTNVWLESEDEILAKAPNFTREQVKGWKGLFCTDGGWLAAAKAINAIGIFLQDKGVKFGFGDAGTFQQPLFAADGKTCIGLETTDGTKYFADKVVLAAGAWSPTLVDLEDQCVSKAWVFAHIQLTPKEADAYKNVPVVYDGEYGFFFEPDEYGVIKVCDEFPGFSRFKLHQPYGAASPKMISVPRSHAKHPTDTYPDASEVTIRKAIARFLPEFKDKELFNRTMCWCTDTADANLLICEHPKWKNFILATGDSGHSFKLLPNIGKYVVELLEGSLSQEMAGAWRWRPGGDALRSRRGAPAKDLAEMPGWKHDAHL

SEQ ID NO: 45 - DNA, 1314 bp, Eupenicillium terrenum
atggctcattcgcgtgcaagcaccaaagtcgtcgtggttgggggaggtggtacgatcgggtcttcgacggctctgcacttaatccgctctggatataccccctcaaatatcaccgtgcttgacgtatacaagaccccttcattgcaatctgcaggacatgatttgaacaagatcatgggcattcgattgcgcaacgggcctgacttgcagctttcgctggaatcactcgacatgtggcaaaacgatgagttgttcaagccattctttcaccaagtgggcatgattgattgttcgtcatccaaagagggtattgaaaatcttcgacgaaaataccagaccctcctcgatgcgggcattgggctggagaagacgaacgtttggctggaatctgaagatgagatcctcgccaaagcgccgaatttcacgcgtgaacaagtcaaggggtggaaaggcttattttgcactgatggaggctggcttgctgcagccaaggctatcaatgcgatcggaattttcctccaggacaaaggtgtcaagtttggctttggagatgctggtacctttcagcaacctctgttcgccgctgatggaaaaacttgcatcggacttgaaactacagacggaaccaagtactttgctgacaaggttgtcttggctgctggtgcgtggagtcccaccttggtggatctagaagatcagtgtgtttcaaaggcctgggttttcgctcatattcaactcacacccaaagaagcggacgcgtacaagaatgtgcctgtggtctatgatggtgaatatgggttctttttcgaacccgacgagtatggggtgatcaaagtctgtgacgagttccctggtttctctcgcttcaaactgcatcaaccgtacggggctgcatctcccaagatgatatccgtaccgcgatcacacgccaagcatcccacagatacctaccctgatgcctccgaagtcaccatacgcaaagcgatcgcaaggttcctgccagaatttaaagacaaggagctcttcaaccgtaccatgtgctggtgtacagatacggccgatgctaacttattgatttgcgaacacccgaagtggaagaatttcattctggccactggagatagcggacattccttcaagctgttgccaaacatcgggaaatacgtagttgagcttttagagggatctctatcgcaggaaatggctggtgcctggagatggagacccggaggtgatgctcttagatctagacgcggtgctccggcaaaggatcttgctgagatgccgggatggaagcatgatgcacatttgtga

SEQ ID NO: 46 - DNA, 30 bp, Artificial
  primer
gactttgatcaccccatactcgtcgggctc

SEQ ID NO: 47 - DNA, 30 bp, Artificial
  primer
ggtgatcaaagtccaggacgagttccctgg

SEQ ID NO: 48 - DNA, 30 bp, Artificial
  primer
ggtgatcaaagtcagtgacgagttccctgg

SEQ ID NO: 49 - DNA, 1314 bp, Phaeosphaeria nodorum
atggccccgtcgcgtgctaatacgtcggtcattgtggttggtggtggtggtacgattggctcatctacggctctgcatctggtccgctcaggctataccccgtcgaacgtgacggttctggatgcatacccgattccgagctctcagagcgctggcaacgacctgaataaaatcatgggtgtctctctgcgtaatccggtggatctgcagctggctctggaagcgcgccaaatgtggaacgaagacgaactgttcaagaagtttttccataacaccggccgtctggattgcgcgcacggtgaaaaagatattgccgacctgaagagcggctatcaggctctggtggatgcgggtctggacgccacgaacgaatggctggatagtgaagacgaaatcctgaaacgtatgccgctgctgtcccgcgatcaaattaaaggctggaaggcgatcttttcaaaagacggtggttggctggcagcagcaaaggcaattaatgcagttggtgaatatctgcgtgatcagggcgtccgcttcggtttttacggcgccggttctttcaaagcaccgctgctggctgaaggcgtctgcatcggtgtcgaaaccgtggatggcacgcgctattacgcagacaaagtggttctggctgcaggtgcatggtcgccgaccctggttgaactgcatgaacagtgtgtgagcaaagcgtgggtttacggccacattcaactgacgccggaagaagccgcacgttataagaacagcccggtcgtgtacaatggcgatgtgggctttttctttgaaccgaacgaacatggcgttatcaaagtctgcgatgaatttccgggttttacccgcttcaagatgcaccagccgtttggtgccaaagcaccgaagcgtattagtgtgccgcgctcccatgccaaacacccgaccgatacgatcccggatgcaagtgacgtttccattcgtcgcgctatcgcgacctttatgccgcagttcaagaacaaaaagatgttcaaccaagcgatgtgctggtgtaccgatacggccgacgctgcgctgctgatttgtgaacatccggaatggaaaaactttgttctggcgaccggcgattcaggtcattcgttcaaactgctgccgaatatcggcaagcacgttgtcgaactgctggagggtacgctggcagatgacctggcacacgcatggcgttggcgtccgggtagtggtgatgcactgaaaagccgtcgctctgctccggcgaaagacctggctgatatgccgggctggaaccatgacaaaccgcgtgctaatctgtaa

SEQ ID NO: 50 - DNA, 30 bp, Artificial
  primer
gactttgataacgccatgttcgttcggttc

SEQ ID NO: 51 - DNA, 30 bp, Artificial
  primer
cgttatcaaagtccaggatgaatttccggg

SEQ ID NO: 52 - DNA, 30 bp, Artificial
  primer
cgttatcaaagtcagcgatgaatttccggg

SEQ ID NO: 53 - protein, 438 aa, Aspergillus nidulans
MTPRANTKIIVVGGGGTMGSSTALHLLRAGYTPSNITVLDTCPIPSAQSAGYDLNKIMGIRLRNKPDLQLSLEALDMWKNDPLFKPFFHNVGMIDVSSTEEGIEGLRKKYQSLLDAGIGLEKTNFMLESEDEILAKAPHFTQEQIKGWKGLFCGDGGWLAAAKAINAIGQFLKEQGVKFGFGGAGTFKKPLFADAHEKTCIGVETVDGTKYYADKVVLAAGAWSSTLVDLEEQCVSKAWVFAHIQLTPAEAAAYKNTPVIYDGDYGFFFEPNENGIIKVCDEFPGFTHFKMHQPYGSPAPKPISVPRSHAKHPTDTYPHASEVTIKKAINRFLPRFNDKELFNRAMCWCTDTADANLLVCEHPRWKGFYLATGDSGHSFKLLPNIGKHVVELLEERLESVFKDAWRWRPGSGDALKSRRAAPAKDLADMPGWRNEAKM

SEQ ID NO: 54 - DNA, 1317 bp, Aspergillus nidulans
atgacgccccgagccaacaccaaaatcattgtcgtcggcggcggcggcacaatgggctcgtcgacagccctacacctcctgcgcgccggctacacgccgtccaacattacagtgctcgacacgtgccctatcccctccgcacagtctgcaggctacgacctgaacaaaatcatggggatccgtctgcgcaacaagcctgatttacagctctctcttgaggcgctggacatgtggaaaaatgatcctctcttcaagccgtttttccacaatgttggaatgatcgacgtctcttcaacagaggaaggcatcgagggtcttcggaagaaataccagtctcttctcgacgcaggcattgggctcgagaagacgaatttcatgctggaaagtgaagacgagatcctggctaaagcgccgcatttcacgcaggagcagattaaaggctggaaaggcctgttctgtggcgacggcggctggctcgctgcagccaaagccatcaatgccattgggcagttcctcaaggaacagggcgtcaagtttggattcggcggcgccggcacgttcaaaaagccactcttcgccgatgcccacgagaagacgtgcatcggcgtcgagactgtagacggcacaaagtactacgccgacaaggtcgttctagcagctggtgcctggagttcgacgttggtcgatctggaggagcagtgcgtttcaaaggcctgggtctttgcccacatccaactgacgcccgctgaagcagccgcgtataagaacactcctgttatatacgacggtgactatgggtttttctttgagccgaatgaaaacggcatcataaaagtctgtgacgaattccctggcttcacgcatttcaaaatgcaccagccgtacggctcgccggcgcccaaacccatctctgtgcctcgttcccatgcgaagcaccccacagatacatacccgcacgcgtcggaggtcacgatcaaaaaggctatcaaccggttcctgccgaggttcaatgacaaggaactgtttaacagggccatgtgctggtgcaccgataccgcggatgcaaatctgcttgtttgtgagcatccacgctggaaggggttttatcttgcaacaggggacagtgggcattcgttcaagttgctgccgaatattggaaagcatgttgtcgagttattggaggagaggctggaaagtgtgtttaaggatgcttggaggtggaggcctggcagtggggatgcattaaaaagtagacgggctgcgcctgcgaaggacctggcggatatgccggggtggaggaatgaggcaaagatgtag

SEQ ID NO: 55 - DNA, 30 bp, Artificial
  primer
gacttttatgatgccgttttcattcggctc

SEQ ID NO: 56 - DNA, 30 bp, Artificial
  primer
catcataaaagtccaggacgaattccctgg

SEQ ID NO: 57 - DNA, 30 bp, Artificial
  primer
catcataaaagtcagtgacgaattccctgg

SEQ ID NO: 58 - DNA, 1323 bp, Curvularia clavata
atggccccgagtcgcgctaacacgagcgtcattgtggtgggtggtggtggcacgattggttcctcaacggcactgcatctggtccgtagcggctataccccgtctaacattaccgtgctggacacgtacccgatcccgagcgcccagtctgcaggcaacgatctgaataaaattatgggtatccgtctgcgcaacaaagttgatctgcagctgtcactggaagcccgtcaaatgtggcgcgaagatgacctgtttaaagaatacttccataacaccggccgtctggattgcgcacacggtgaagaaggtctggccgacctgcgccaggcttaccaagcgctgctggatgccaacgcaggtctggaagaaaccacggaatggctggattcagaagacgaaattctgaagaaaatgccgctgctggatcgtgaacagatcaaaggttggaaagccgtgtattcgcaagatggcggttggctggcggccgcaaaagccattaatgcaatcggcgaatacctgcgcgcgcagggcgttaaattcggttttggcggtgctggttcctttaaacagccgctgctggcagaaggcgtctgcattggtgtcgaaaccgtggatggcacgcgttattacgcggacaaagtggttctggctgcaggtgcatggagtccggtgctggttgatctggaagaccagtgtgtgtccaaagcgtgggtttatgcgcatatccaactgaccccggaagaagccgcagaatataaaaacgtcccggtcgtgtacaatggcgatgtgggctttttctttgaaccggacgaacatggcgttattaaagtctgcgatgaatttccgggttttacccgcttcaaacagcaccaaccgtatggcgctaaagcgccgaaacgtatctcagtgccgcgttcggctgcaaaacacccgaccgatacgtacccggacgcgagtgaaaaatccattcgtaaagccatcgcaacctttctgccgaaattcacggaaaaagaactgtttaatcgccatctgtgctggtgtaccgatacggccgacgccgcactgctgatgtgtgaacacccggaatggaaaaactttgttctggcgaccggcgatagcggtcatacgttcaaactgctgccgaatattggcaaacacgttgtcgaactgctggaaggtaccctggcagaagacctggctcatgcgtggcgttggcgtccgggtacgggtgatgcactgaaatctcgtcgcgctgcgccggcgaaagacctggcggatatgccgggctggaaacacgacgatgtggtgaaaagcaaactgtaa

SEQ ID NO: 59 - DNA, 30 bp, Artificial
  primer
gactttaataacgccatgttcgtccggttc

SEQ ID NO: 60 - DNA, 29 bp, Artificial
  primer
cgttattaaagtccaggatgaatttccgg

SEQ ID NO: 61 - DNA, 29 bp, Artificial
  primer
cgttattaaagtcagcgatgaatttccgg

SEQ ID NO: 62 - DNA, 30 bp, Artificial
  primer
gcccacatcgccattgtacacgaccgggac

SEQ ID NO: 63 - DNA, 30 bp, Artificial
  primer
ttattctttgaaccggacgaacatggcgtt

SEQ ID NO: 64 - DNA, 30 bp, Artificial
  primer
atgttctttgaaccggacgaacatggcgtt

SEQ ID NO: 65 - DNA, 30 bp, Artificial
  primer
gaaaaagcccacatcgccattgtacacgac

SEQ ID NO: 66 - DNA, 30 bp, Artificial
  primer
ttagaaccggacgaacatggcgttattaaa

SEQ ID NO: 67 - protein, 438 aa, Emericella nidulans
MAPRANTKIIVVGGGGTMGSSTALHLLRAGYTPSNITVLDTYPIPSAQSAGYDLNKIFGISGANKHDLQLSLEAFDMWKNDPLFKPFFHNVGQMDVSSTEEGIKRLRRRYQSLLRAGIGLEKTNFLLESEDEILAKAPHFTREQIKGWKGLFCGDGGWLAAAKAINAIGQFLKEQGVKFGFGEAGTFKKPLFADADEKTCIGVETVDGTKYYADKVVLAAGAWSSTLVDLEEQCVSKAWVFAHIQLTPAEAAAYKNTPVIYDGDYGFFIEPDENGIIKVCDEFPGFTHFKMHQPYGSPVPKLISVPRSHAKHPTDTYPHASEVTIKKAINRFLPRFNDKELFNRAMCWCTDTADSNLLVCEHPRWKGFYLATGDSGHSFKLLPNIGKHVVELLEGRLESVFKDAWRWRPGSGDALKSRRAAPAKDLADMPGWRNEAKM

SEQ ID NO: 68 - DNA, 1317 bp, Emericella nidulans
atggctccgcgtgcgaatacgaaaatcattgttgtcggtggtggtggtacgatgggttcaagtacggctctgcatctgctgcgtgcgggctataccccgagcaacattaccgtgctggatacgtatccgatcccgtcagcgcagtcggccggttacgacctgaacaaaatttttggtatcagcggtgcaaataaacatgatctgcaactgtctctggaagcgtttgatatgtggaaaaacgacccgctgtttaaaccgtttttccacaatgtgggccagatggatgttagctctaccgaagaaggtattaaacgcctgcgtcgccgttaccaaagtctgctgcgtgccggcatcggtctggaaaaaaccaacttcctgctggaatccgaagatgaaattctggcgaaagccccgcatttcacgcgcgaacagatcaaaggctggaaaggtctgttttgcggtgatggcggttggctggccgcagcaaaagcaattaatgctatcggccagtttctgaaagaacaaggtgtgaaatttggcttcggtgaagcgggtaccttcaaaaaaccgctgtttgcagatgctgacgaaaaaacgtgcattggcgttgaaaccgtcgatggtacgaaatattacgcagacaaagtggttctggctgcgggcgcttggagttccaccctggttgatctggaagaacagtgtgtcagcaaagcgtgggtgtttgcccacatccaactgaccccggccgaagccgcagcttataaaaacacgccggtgatttatgatggcgactacggctttttcatcgaaccggatgaaaatggcattatcaaagtttgcgacgaatttccgggtttcacccattttaaaatgcaccagccgtatggctcaccggttccgaaactgattagtgtcccgcgttcccatgcaaaacacccgaccgatacgtacccgcatgcatcggaagtcacgattaagaaagcgatcaaccgcttcctgccgcgttttaacgacaaagaactgttcaatcgcgcgatgtgctggtgtaccgatacggccgacagcaatctgctggtttgtgaacacccgcgttggaaaggtttctatctggcgaccggcgatagcggtcattcttttaaactgctgccgaatattggcaaacacgtcgtggaactgctggaaggtcgcctggaatctgtgtttaaagatgcgtggcgctggcgtccgggctcaggtgatgcactgaaatcgcgtcgcgcagcaccggcgaaagacctggcggatatgccgggttggcgtaatgaagcgaaaatgtaa

SEQ ID NO: 69 - DNA, 35 bp, Artificial
  primer
gaaggagatatacatatggctccgcgtgcgaatac

SEQ ID NO: 70 - DNA, 35 bp, Artificial
  primer
ctcgaattcggatccttacattttcgcttcattac

SEQ ID NO: 71 - DNA, 30 bp, Artificial
  primer
ggatccgaattcgagctccgtcgacaagct

SEQ ID NO: 72 - DNA, 30 bp, Artificial
  primer
atgtatatctccttcttaaagttaaacaaa

SEQ ID NO: 73 - DNA, 30 bp, Artificial
  primer
aactttgataatgccattttcatccggttc

SEQ ID NO: 74 - DNA, 30 bp, Artificial
  primer
caggacgaatttccgggtttcacccatttt

SEQ ID NO: 75 - DNA, 30 bp, Artificial
  primer
agcgacgaatttccgggtttcacccatttt

SEQ ID NO: 76 - DNA, 30 bp, Artificial
  primer
gccgtagtcgccatcataaatcaccggcgt

SEQ ID NO: 77 - DNA, 30 bp, Artificial
  primer
ttattcatcgaaccggatgaaaatggcatt

SEQ ID NO: 78 - DNA, 30 bp, Artificial
  primer
atgttcatcgaaccggatgaaaatggcatt

SEQ ID NO: 79 - DNA, 30 bp, Artificial
  primer
gaaaaagccgtagtcgccatcataaatcac

SEQ ID NO: 80 - DNA, 30 bp, Artificial
  primer
ctcgaaccggatgaaaatggcattatcaaa

SEQ ID NO: 81 - DNA, 30 bp, Artificial
  primer
atggaaccggatgaaaatggcattatcaaa

SEQ ID NO: 82 - DNA, 30 bp, Artificial
  primer
atggaaccggacgaacatggcgttattaaa